European Patent Application EP 4 198 048 A1, published June 21, 2023. Title: CALPAIN-3 GENE TRANSFER INCREASE USING MODIFIED ITR SEQUENCES. Applicant: GENETHON INSTITUT NATIONAL DE LA SANTE ET DE LA RECHERCHE MEDICALE UNIVERSITE D'EVRY VAL D’ESSONNE. The sequence listing filed with the application follows.

SEQUENCE LISTING (6 sequences)

SEQ ID NO: 1 - DNA, 130 bp, Artificial Sequence
  ITRg 5' flop
ctgcgcgctcgctcgctcactgaggccgcccgggcaaagcccgggcgtcgggcgacctttggtcgcccggcctcagtgagcgagcgagcgcgcagagagggagtggccaactccatcactaggggttcct

SEQ ID NO: 2 - DNA, 130 bp, Artificial Sequence
  ITRg 3' 130 bp
aggaacccctagtgatggagttggccactccctctctgcgcgctcgctcgctcactgaggccgggcgaccaaaggtcgcccgacgcccgggctttgcccgggcggcctcagtgagcgagcgagcgcgcag

SEQ ID NO: 3 - DNA, 128 bp, Artificial Sequence
  ITRg 3' flip 128 bp
aggaacccctagtgatggagttggccactccctctctgcgcgctcgctcgctcactgaggccgggcgaccaaaggtcgcccgacgcccgggctttgcccgggcggcctcagtgagcgagcgagcgcgc

SEQ ID NO: 4 - DNA, 2466 bp, Artificial Sequence
  calpain
atgccgaccgtcattagcgcatctgtggctccaaggacagcggctgagccccggtccccagggccagttcctcacccggcccagagcaaggccactgaggctgggggtggaaacccaagtggcatctattcagccatcatcagccgcaattttcctattatcggagtgaaagagaagacattcgagcaacttcacaagaaatgtctagaaaagaaagttctttatgtggaccctgagttcccaccggatgagacctctctcttttatagccagaagttccccatccagttcgtctggaagagacctccggaaatttgcgagaatccccgatttatcattgatggagccaacagaactgacatctgtcaaggagagctaggggactgctggtttctcgcagccattgcctgcctgaccctgaaccagcaccttcttttccgagtcataccccatgatcaaagtttcatcgaaaactacgcagggatcttccacttccagttctggcgctatggagagtgggtggacgtggttatagatgactgcctgccaacgtacaacaatcaactggttttcaccaagtccaaccaccgcaatgagttctggagtgctctgctggagaaggcttatgctaagctccatggttcctacgaagctctgaaaggtgggaacaccacagaggccatggaggacttcacaggaggggtggcagagttttttgagatcagggatgctcctagtgacatgtacaagatcatgaagaaagccatcgagagaggctccctcatgggctgctccattgatgatggcacgaacatgacctatggaacctctccttctggtctgaacatgggggagttgattgcacggatggtaaggaatatggataactcactgctccaggactcagacctcgaccccagaggctcagatgaaagaccgacccggacaatcattccggttcagtatgagacaagaatggcctgcgggctggtcagaggtcacgcctactctgtcacggggctggatgaggtcccgttcaaaggtgagaaagtgaagctggtgcggctgcggaatccgtggggccaggtggagtggaacggttcttggagtgatagatggaaggactggagctttgtggacaaagatgagaaggcccgtctgcagcaccaggtcactgaggatggagagttctggatgtcctatgaggatttcatctaccatttcacaaagttggagatctgcaacctcacggccgatgctctgcagtctgacaagcttcagacctggacagtgtctgtgaacgagggccgctgggtacggggttgctctgccggaggctgccgcaacttcccagatactttctggaccaaccctcagtaccgtctgaagctcctggaggaggacgatgaccctgatgactcggaggtgatttgcagcttcctggtggccctgatgcagaagaaccggcggaaggaccggaagctaggggccagtctcttcaccattggcttcgccatctacgaggttcccaaagagatgcacgggaacaagcagcacctgcagaaggacttcttcctgtacaacgcctccaaggcccgtagcaaaacctacatcaacatgagagaggtgagccagcgcttccgcctgcctcccagcgagtacgtcatcgtgccctccacctacgagccccaccaggagggggaattcatcctccgggtcttctctgaaaagaggaacctctctgaggaagttgaaaataccatctccgtggatcggccagtgaaaaagaaaaaaaccaagcccatcatcttcgtttcggacagagcaaacagcaacaaggagctgggtgtggaccaggagtcagaggagggcaaaggcaaaacaagccctgataagcaaaagcagtccccacagccacagcctggcagctctgatcaggaaagtgaggaacagcaacaattccggaacattttcaagcagatagcaggagatgacatggagatctgtgcagatgagctcaagaaggtccttaacacagtcgtgaacaaacacaaggacctgaagacacacgggttcacactggagtcctgccgtagcatgattgcgctcatggatacagatggctctggaaagctcaacctgcaggagttccaccacctctggaacaagattaaggcctggcagaaaattttcaaacactatgacacagaccagtccggcaccatcaacagctacgagatgcgaaatgcagtcaacgacgcaggattccacctcaacaaccagctctatgacatcattaccatgcggtacgcagacaaacacatgaacatcgactttgacagtttcatctgctgcttcgttaggctggagggcatgttcagagcttttcatgcatttgacaaggatggagatggtatcatcaagctcaacgttctggagtggctgcagctcaccatgtatgcctga

SEQ ID NO: 5 - DNA, 1061 bp, Artificial Sequence
  Human Desmin Promoter
taccccctgccccccacagctcctctcctgtgccttgtttcccagccatgcgttctcctctataaatacccgctctggtatttggggttggcagctgttgctgccagggagatggttgggttgacatgcggctcctgacaaaacacaaacccctggtgtgtgtgggcgtgggtggtgtgagtagggggatgaatcagggagggggcgggggacccagggggcaggagccacacaaagtctgtgcgggggtgggagcgcacatagcaattggaaactgaaagcttatcagaccctttctggaaatcagcccactgtttataaacttgaggccccaccctcgacagtaccggggaggaagagggcctgcactagtccagagggaaactgaggctcagggctagctcgcccatagacatacatggcaggcaggctttggccaggatccctccgcctgccaggcgtctccctgccctcccttcctgcctagagacccccaccctcaagcctggctggtctttgcctgagacccaaacctcttcgacttcaagagaatatttaggaacaaggtggtttagggcctttcctgggaacaggccttgaccctttaagaaatgacccaaagtctctccttgaccaaaaaggggaccctcaaactaaagggaagcctctcttctgctgtctcccctgaccccactcccccccaccccaggacgaggagataaccagggctgaaagaggcccgcctgggggctgcagacatgcttgctgcctgccctggcgaaggattggcaggcttgcccgtcacaggacccccgctggctgactcaggggcgcaggcctcttgcgggggagctggcctccccgcccccacggccacgggccgccctttcctggcaggacagcgggatcttgcagctgtcaggggaggggaggcgggggctgatgtcaggagggatacaaatagtgccgacggctgggggccctgtctcccctcgccgcatccactctccggccggccgcctgcccgccgcctcctccgtgcgcccgccagcctcgcccgc

SEQ ID NO: 6 - DNA, 762 bp, Artificial Sequence
  pA-HBB2
accccaccagtgcaggctgcctatcagaaagtggtggctggtgtggctaatgccctggcccacaagtatcactaagctcgctttcttgctgtccaatttctattaaaggttcctttgttccctaagtccaactactaaactgggggatattatgaagggccttgagcatctggattctgcctaataaaaaacatttattttcattgcaatgatgtatttaaattatttctgaatattttactaaaaagggaatgtgggaggtcagtgcatttaaaacataaagaaatgaagagctagttcaaaccttgggaaaatacactatatcttaaactccatgaaagaaggtgaggctgcaaacagctaatgcacattggcaacagccctgatgcctatgccttattcatccctcagaaaaggattcaagtagaggcttgatttggaggttaaagttttgctatgctgtattttacattacttattgttttagctgtcctcatgaatgtcttttcactacccatttgcttatcctgcatctctcagccttgactccactcagttctcttgcttagagataccacctttcccctgaagtgttccttccatgttttacggcgagatggtttctcctcgcctggccactcagccttagttgtctctgttgtcttatagaggtctacttgaagaaggaaaaacagggggcatggtttgactgtcctgtgagcccttcttccctgcctcccccactcacagtgacccggaatc